European Patent Specification EP 4 056 700 B1, published June 3, 2026. Title: rAAV-Guanylate Cyclase Compositions and Methods for Treating Leber's Congenital Amaurosis-1 (LCA1). Applicant: University of Florida Research Foundation, Inc. Boye, Shannon E. Hauswirth, William W. Boye, Sanford L. The sequence listing filed with the application follows.

SEQUENCE LISTING (18 sequences)

SEQ ID NO: 1 - protein, 1103 aa, Homo sapiens
MTACARRAGGLPDPGLCGPAWWAPSLPRLPRALPRLPLLLLLLLLQPPALSAVFTVGVLGPWACDPIFSRARPDLAARLAAARLNRDPGLAGGPRFEVALLPEPCRTPGSLGAVSSALARVSGLVGPVNPAACRPAELLAEEAGIALVPWGCPWTQAEGTTAPAVTPAADALYALLRAFGWARVALVTAPQDLWVEAGRSLSTALRARGLPVASVTSMEPLDLSGAREALRKVRDGPRVTAVIMVMHSVLLGGEEQRYLLEAAEELGLTDGSLVFLPFDTIHYALSPGPEALAALANSSQLRRAHDAVLTLTRHCPSEGSVLDSLRRAQERRELPSDLNLQQVSPLFGTIYDAVFLLARGVAEARAAAGGRWVSGAAVARHIRDAQVPGFCGDLGGDEEPPFVLLDTDAAGDRLFATYMLDPARGSFLSAGTRMHFPRGGSAPGPDPSCWFDPNNICGGGLEPGLVFLGFLLVVGMGLAGAFLAHYVRHRLLHMQMVSGPNKIILTVDDITFLHPHGGTSRKVAQGSRSSLGARSMSDIRSGPSQHLDSPNIGVYEGDRVWLKKFPGDQHIAIRPATKTAFSKLQELRHENVALYLGLFLARGAEGPAALWEGNLAVVSEHCTRGSLQDLLAQREIKLDWMFKSSLLLDLIKGIRYLHHRGVAHGRLKSRNCIVDGRFVLKITDHGHGRLLEAQKVLPEPPRAEDQLWTAPELLRDPALERRGTLAGDVFSLAIIMQEVVCRSAPYAMLELTPEEVVQRVRSPPPLCRPLVSMDQAPVECILLMKQCWAEQPELRPSMDHTFDLFKNINKGRKTNIIDSMLRMLEQYSSNLEDLIRERTEELELEKQKTDRLLTQMLPPSVAEALKTGTPVEPEYFEQVTLYFSDIVGFTTISAMSEPIEVVDLLNDLYTLFDAIIGSHDVYKVETIGDAYMVASGLPQRNGQRHAAEIANMSLDILSAVGTFRMRHMPEVPVRIRIGLHSGPCVAGVVGLTMPRYCLFGDTVNTASRMESTGLPYRIHVNLSTVGILRALDSGYQVELRGRTELKGKGAEDTFWLVGRRGFNKPIPKPPDLQPGSSNHGISLQEIPPERRRKLEKARPGQFS

SEQ ID NO: 2 - protein, 1108 aa, Mus musculus
MSAWLLPAGGLPGAGFCVPARQSPSSFSRVLRWPRPGLPGLLLLLLLPSPSALSAVFKVGVLGPWACDPIFARARPDLAARLAANRLNRDFALDGGPRFEVALLPEPCLTPGSLGAVSSALSRVSGLVGPVNPAACRPAELLAQEAGVALVPWGCPGTRAAGTTAPAVTPAADALYVLLRAFRWARVALITAPQDLWVEAGRALSTALRARGLPVALVTSMETSDRSGAREALGRIRDGPRVRVVIMVMHSVLLGGEEQRYLLEAAEELALTDGSLVFLPFDTLHYALSPGPEALAAFVNSSQLRRAHDAVLTLTRRCPPGGSVQDSLRRAQEHQELPLDLNLKQVSPLFGTIYDAVFLLAGGVKRARTAVGGGWVSGASVARQVREAQVSGFCGVLGRTEEPSFVLLDTDASGEQLFATHLLDPVLGSLRSAGTPMHFPRGGPAPGPDPSCWFDPDVICNGGVEPGLVFVGFLLVIGMGLTGAFLAHYLRHRLLHMQMASGPNKIILTLEDVTFLHPPGGSSRKVVQGSRSSLATRSASDIRSVPSQPQESTNVGLYEGDWVWLKKFPGEHHMAIRPATKTAFSKLRELRHENVALYLGLFLAGTADSPATPGEGILAVVSEHCARGSLHDLLAQREIKLDWMFKSSLLLDLIKGMRYLHHRGVAHGRLKSRNCVVDGRFVLKVTDHGHGRLLEAQRVLPEPPSAEDQLWTAPELLRDPSLERRGTLAGDVFSLAIIMQEVVCRSTPYAMLELTPEEVIQRVRSPPPLCRPLVSMDQAPMECIQLMTQCWAEHPELRPSMDLTFDLFKSINKGRKTNIIDSMLRMLEQYSSNLEDLIRERTEELEQEKQKTDRLLTQMLPPSVAEALKMGTSVEPEYFEEVTLYFSDIVGFTTISAMSEPIEVVDLLNDLYTLFDAIIGAHDVYKVETIGDAYMVASGLPQRNGQRHAAEIANMSLDILSAVGSFRMRHMPEVPVRIRIGLHSGPCVAGVVGLTMPRYCLFGDTVNTASRMESTGLPYRIHVNMSTVRILRALDQGFQMECRGRTELKGKGIEDTYWLVGRLGFNKPIPKPPDLQPGASNHGISLQEIPPERRKKLEKARPGQFTGK

SEQ ID NO: 3 - protein, 1108 aa, Rattus norvegicus
MSAWLLPAGGFPGAGFCIPAWQSRSSLSRVLRWPGPGLPGLLLLLLLPSPSAFSAVFKVGVLGPWACDPIFARARPDLAARLATDRLNRDLALDGGPWFEVTLLPEPCLTPGSLGAVSSALTRVSGLVGPVNPAACRPAELLAQEAGVALVPWGCPGTRAAGTTAPAVTPAADALYVLLKAFRWARVALITAPQDLWVEAGRALSTALRARGLPVALVTSMVPSDLSGAREALRRIRDGPRVRVVIMVMHSVLLGGEEQRYLLEAAEELGLTDGSLVFLPFDTLHYALSPGPEALAAFVNSSKLRRAHDAVLTLTRRCPPGGSVQDSLRRAQEHQELPLDLDLKQVSPLFGTIYDAVFLLAGGVTRARAAVGGGWVSGASVARQMREAQVFGFCGILGRTEEPSFVLLDTDAAGERLFTTHLLDPVLGSLRSAGTPVHFPRGAPAPGPDPSCWFDPDVICNGGVEPGLVFVGFLLVIVVGLTGAFLAHYLRHRLLHMQMVSGPNKIILTLEDVTFLHPQGGSSRKVAQGSRSSLATRSTSDIRSVPSQPQESTNIGLYEGDWVWLKKFPGEHHMAIRPATKMAFSKLRELRHENVALYLGLFLAGTADSPATPGEGILAVVSEHCARGSLHDLLAQRDIKLDWMFKSSLLLDLIKGMRYLHHRGVAHGRLKSRNCVVDGRFVLKVTDHGHGRLLEAQRVLPEPPSAEDQLWTAPELLRDPALERRGTLAGDVFSLGIIMQEVVCRSTPYAMLELTPEEVIQRVRSPPPLCRPLVSMDQAPMECIQLMAQCWAEHPELRPSMDLTFDLFKGINKGRKTNIIDSMLRMLEQYSSNLEDLIRERTEELEQEKQKTDRLLTQMLPPSVAEALKMGTSVEPEYFEEVTLYFSDIVGFTTISAMSEPIEVVDLLNDLYTLFDAIIGSHDVYKVETIGDAYMVASGLPQRNGQRHAAEIANMSLDILSAVGSFRMRHMPEVPVRIRIGLHSGPCVAGVVGLTMPRYCLFGDTVNTASRMESTGLPYRIHVNMSTVRILRALDQGFQMECRGRTELKGKGVEDTYWLVGRVGFNKPIPKPPDLQPGASNHGISLQEIPPERRKKLEKARPGQFTGK

SEQ ID NO: 4 - protein, 1110 aa, Bos taurus
MTACTFLAGGLRDPGLCAPTRWSPSPPGLPPIPPRPRLRLRPPLLLLLLLPRSVLSAVFTVGVLGPWACDPIFARARPDLAARLAASRLNHAAALEGGPRFEVALLPEPCRTPGSLGAVSSALTRVSGLVGPVNPAACRPAELLAQEAGVALVPWGCPGTRAAGTTAPVVTPAADALYALLRAFRWAHVALVTAPQDLWVEAGHALSTALRARGLPVALVTSMEPSDLSGAREALRRVQDGPRVRAVIMVMHSVLLGGEEQRCLLEAAEELGLADGSLVFLPFDTLHYALSPGPDALAVLANSSQLRKAHDAVLTLTRHCPLGGSVRDSLRRAQEHRELPLDLNLQQVSPLFGTIYDSVFLLAGGVARARVAAGGGWVSGAAVARHIRDARVPGFCGALGGAEEPSFVLLDTDATGDQLFATYVLDPTQGFFHSAGTPVHFPKGGRGPGPDPSCWFDPDTICNGGVEPSVVFIGFLLVVGMGLAGAFLAHYCRHRLLHIQMVSGPNKIILTLDDITFLHPHGGNSRKVAQGSRTSLAARSISDVRSIHSQLPDYTNIGLYEGDWVWLKKFPGDRHIAIRPATKMAFSKIRELRHENVALYLGLFLAGGAGGPAAPGEGVLAVVSEHCARGSLQDLLAQRDIKLDWMFKSSLLLDLIKGIRYLHHRGVAHGRLKSRNCVVDGRFVLKVTDHGHGRLLEAQRVLPEPPSAEDQLWTAPELLRDPVLERRGTLAGDVFSLGIIMQEVVCRSAPYAMLELTPEEVVKRVQSPPPLCRPSVSIDQAPMECIQLMKQCWAEQPELRPSMDRTFELFKSINKGRKMNIIDSMLRMLEQYSSNLEDLIRERTEELELEKQKTDRLLTQMLPPSVAEALKMGTPVEPEYFEEVTLYFSDIVGFTTISAMSEPIEVVDLLNDLYTLFDAIIGSHDVYKVETIGDAYMVASGLPQRNGHRHAAEIANMALDILSAVGTFRMRHMPEVPVRIRIGLHSGPCVAGVVGLTMPRYCLFGDTVNTASRMESTGLPYRIHVNRSTVQILSALNEGFLTEVRGRTELKGKGAEETYWLVGRRGFNKPIPKPPDLQPGASNHGISLHEIPPDRRQKLEKARPGQFSGK

SEQ ID NO: 5 - protein, 1109 aa, Canis familiaris
MSACALLAGGLPDPRLCAPARWARSPPGVPGAPPWPQPRLRLLLLLLLLPPSALSAVFTVGVLGPWACDPIFARARPDLAARLAAARLNRDAALEDGPRFEVTLLPEPCRTPGSLGAVSSALGRVSGLVGPVNPAACRPAELLAQEAGVALVPWSCPGTRAGGTTAPAGTPAADALYALLRAFRWARVALITAPQDLWVEAGRALSAALRARGLPVALVTTMEPSDLSGAREALRRVQDGPRVRAVIMVMHSVLLGGEEQRCLLQAAEELGLADGSLVFLPFDTLHYALSPGPEALAVLANSSQLRRAHDAVLILTRHCPPGGSVMDNLRRAQEHQELPSDLDLQQVSPFFGTIYDAVLLLAGGVARARAAAGGGWVSGATVAHHIPDAQVPGFCGTLGGAQEPPFVLLDTDAAGDRLFATYMLDPTRGSLLSAGTPVHFPRGGGTPGSDPSCWFEPGVICNGGVEPGLVFLGFLLVVGMGLTGAFLAHYLRHRLLHIQMVSGPNKIILTLDDVTFLHPHGGSTRKVVQGSRSSLAARSTSDIRSVPSQPLDNSNIGLFEGDWVWLKKFPGDQHIAIRPATKTAFSKLRELRHENVVLYLGLFLGSGGAGGSAAGEGVLAVVSEHCARGSLHDLLAQRDIKLDWMFKSSLLLDLIKGMRYLHHRGVAHGRLKSRNCVVDGRFVLKVTDHGHARLMEAQRVLLEPPSAEDQLWTAPELLRDPALERRGTLPGDVFSLGIIMQEVVCRSAPYAMLELTPEEVVERVRSPPPLCRPSVSMDQAPVECIQLMKQCWAEHPDLRPSLGHIFDQFKSINKGRKTNIIDSMLRMLEQYSSNLEDLIRERTEELELEKQKTDRLLTQMLPPSVAEALKMGTPVEPEYFEEVTLYFSDIVGFTTISAMSEPIEVVDLLNDLYTLFDAIIGSHDVYKVETIGDAYMVASGLPQRNGQRHAAEIANMALDILSAVGSFRMRHMPEVPVRIRIGLHSGPCVAGVVGLTMPRYCLFGDTVNTASRMESTGLPYRIHVNMSTVRILHALDEGFQTEVRGRTELKGKGAEDTYWLVGRRGFNKPIPKPPDLQPGASNHGISLQEIPLDRRWKLEKARPGQFSGK

SEQ ID NO: 6 - protein, 1103 aa, Macaca mulatta
MTACARRAGGLPDPRLCGPARWAPALPRLPRALPRLPLLLLLLLLQPPALSAVFTVGVLGPWACDPIFSRARADLAARLAAARLNRDPDLAGGPRFEVALLPEPCRTPGSLGAVSSALTRVSGLVGPVNPAACRPAELLAEEAGIALVPWGCPGTQAAGTTAPALTPAADALYALLRAFGWARVALVTAPQDLWVEAGHSLSTALRARGLPVASVTSMEPLDLSGAREALRKVRDGPRVTAVIMVMHSVLLGGEEQRYLLEAAEELGLTDGSLVFLPFDTVHYALSPGPEALAALANSSQLRRAHDAVLTLTRHCPSEGSVLDSLRRAQERRELPSDLNLQQVSPLFGTIYDAVFLLVRGVAEARAAAGGRWVSGAAVARHVWDAQVPGFCGDLGGDEEPPFVLLDTDAVGDRLFATYMLDPTRGSLLSAGTPMHFPRGGSAPGPDPSCWFDPNNICGGGLEPGLVFLGFLLVVGMGLAGAFLAHYVRHQLLHIQMVSGPNKIILTVDDITFLHPHGGTSRKVAQGSRSSLAARSMSDVRSGPSQPTDSPNVGVYEGDRVWLKKFPGDQHIAIRPATKTAFSKLQELRHENVALYLGLFLAQGAEGPAALWEGNLAVVSEHCTRGSLQDLLAQREIKLDWMFKSSLLLDLIKGIRYLHHRGVAHGRLKSRNCIVDGRFVLKITDHGHGRLLEAQKVLPEPPRAEDQLWTAPELLRDPALERRGTLAGDVFSLAIIMQEVVCRSAPYAMLELTPEEVVQRVRSPPPLCRPLVSMDQAPVECIHLMKQCWAEQPELRPSMDHTFDLFKNINKGRKTNIIDSMLRMLEQYSSNLEDLIRERTEELELEKQKTDRLLTQMLPPSVAEALKTGTPVEPEYFEQVTLYFSDIVGFTTISAMSEPIEVVDLLNDLYTLFDAIIGSHDVYKVETIGDAYMVASGLPQRNGQRHAAEIANMSLDILSAVGTFRMRHMPEVPVRIRIGLHSGPCVAGVVGLTMPRYCLFGDTVNTASRMESTGLPYRIHVNLSTVGILRALDSGYQVELRGRTELKGKGAEDTFWLVGRRGFNKPIPKPPDLQPGSSNHGISLQEIPPERRRKLEKARPGQFS

SEQ ID NO: 7 - protein, 1103 aa, Pongo pygmaeus
MTACARRAGGLPDPGLCGPARWAPSLPRLPRALPRLPLLLLLLLLQPPALSAVFTVGVLGPWACDPIFSRARPDLAARLAAARLNRDPGLAGGPRFEVALLPEPCRTPGSLGAVSSALARVSGLVGPVNPAACRPAELLADNPGIALVPWGCPWTQAEGTTAPCVTPAADALYALLRAFGWARVALVTAPQDLWVEAGRSLSTALRARGLPVASVTSMEPLDLSGAREALRKVRDGPRVTAVIMVMHSVLLGGEEQRYLLEAAEELGLTDGSLVFLPFDTIHYALSPGPEALAALANSSQLRRAHDAVLTLTRHCPSEGSVLDSLRRAQERRELPSDLNLQQVSPLFGTIYDAVFLLARGVAEAWAAAGGRWVSGAAVARHIRDAQVPGFCGDLGGDGEPPFVLLDTDAAGDRLFATYMLDPARGSFLSAGTRMHFPRGGSAPGPDPSCWFDPNNICGGGLEPGLVFLGFLLVVGMGLAGAFLAHYVRHRLLHIQMVSGPNKIILTVNDITFLHPHGGTSRKVAQGSRSSLAARSMSDIRSGPSQPLDSPNVGVYEGDRVWLKKFPGDQHIAIRPATKTAFSKLQELRHENVALYLGLFLARGAEGPAALWEGNLAVVSEHCTRGSLQDLLSQREIKLDWMFKSSLLLDLIKGIRYLHHRGVAHGRLKSRNCIVDGRFVLKITDHGHGRLLEAQKVLPEPPRAEDQLWTAPELLRDPALERRGTLAGDVFSLAIIMQEVVCRSAPYAMLELTPEEVVQRVRSPPPLCRPLVSMDQAPVECIHLMKQCWAEQPELRPSMDHTFDLFKNINKGRKTNIIDSMLRMLEQYSSNLEDLIRERTEELELEKQKTDRLLTQMLPPSVAEALKTGTPVEPEYFEQVTLYFSDIVGFTTISAMSEPIEVVDLLNDLYTLFDAIIGSHDVYKVETIGDAYMVASGLPQRNGQRHAAEIANMSLDILSAVGTFRMRHMPEVPVRIRIGLHSGPCVAGVVGLTMPRYCLFGDTVNTASRMESTGLPYRIHVNLSTVGILRALDSGYQVELRGRTELKGKGAEDTFWLVGRRGFNKPIPKPPDLQPGSSNHGISLQEIPPERRRKLEKARPGQFS

SEQ ID NO: 8 - protein, 1103 aa, Callithrix jacchus
MTACARRAGGLPDPGLCGPARWAPALSRLPRALPRLPLLLLLLLLQPPALSAQFTVGVLGPWACDPIFSRARPDLAARLAAARLNRDPSLAGGPRFEVALLPEPCRTPGSLGAVSSALARVSGLVGPVNPAACRPAELLAEEAGIALVPWGCPGTQAAGTTAPVVTPAADALYALLRAFGWARVALVTAPQDLWVEAGLSLSTALRARGLPVVSVTSMEPLDLSGAREALRKVRNGPRVTAVIMVMHSVLLGGEEQRYLLEAAEELGLTDGSLVFLPFDTIHYALSPGREALAALVNSSQLRRAHDAVLTLTRHCSSEGSVLDSLRKAQQRRELPSDLNLEQVSPLFGTIYDAVVLLARGVADARAAVGGRWVSGAAVARHVWDAQASGFCGDLGRDEEPSFVLLDTDAAGDQLFATYMLDPARGSLLSAGTPMHFPRGGPAPGPDPSCWFDPNNICDGGLEPGFIFLGFLLVVGMGLAGALLAHYVRHQLLHIQMVSGPNKIILTVDDITFLHPHGGASRKVAQGSRSSLAAHSTSDIRSGPSQPSDSPNIGVYEGDRVWLKKFPGEQHIAIRPATKTAFSKLQELRHENVALYLGLFLAQGAEGPAALWEGNLAVVSEHCTRGSLQDLLAQREIKLDWMFKSSLLLDLIKGIRYLHHRGVAHGRLKSRNCIVDGRFVLKITDHGHGRLLEAQKVLPEPPKAEDQLWTAPELLRDPALERRGTLAGDVFSLGIIMQEVVCRSAPYAMLELTPDEVVQRVRSPPPLCRPFVSMDQAPVECIHLMKQCWAEQPELRPSMDLTFDLFKNINKGRKTNIIDSMLRMLEQYSSNLEDLIRERTEELELEKQKTDRLLTQMLPPSVAEALKTGTPVEPEYFEQVTLYFSDIVGFTTISAMSEPIEVVDLLNDLYTLFDAIIGSHDVYKVETIGDAYMVASGLPQRNGQRHAAEIANMSLDILSAVGTFRMRHMPEVPVRIRIGLHSGPCVAGVVGLTMPRYCLFGDTVNTASRMESTGLPYRIHVNLSTVGILRALDSGYQVELRGRTELKGKGAEDTFWLVGRRGFNKPIPKPPDLQPGASNHGISLQEIPPERRRKLEKARPGQFS

SEQ ID NO: 9 - protein, 1012 aa, Ailuropoda melanoleuca
  misc_feature (80)..(88): Xaa can be any naturally occurring amino acid
  misc_feature (964)..(971): Xaa can be any naturally occurring amino acid
MRACALLAGGLPYPRLCAPTRWAPARPGVSRALPWPRPRLRLLLLLLLRPPSVLSAVFTVGVLGPWACDPIFARARPDLXXXXXXXXXDALYVLLRAFRWARVALVTAPQDLWVEAGRALSAALRARGLPVALVTTMEPSDLSGAREALRRVQHGPRVSAVIMVMHSVLLGGEEQRCLLQAAEELGLADGSLVFLPFDTLHYALSPGPEALAALANSSQLRRAHDAVLTLTRHCPPGGSVMDSLRRAQERQELPSDLNLEQVSPLFGTIYDAVFLLAGGVARARAAAADSRVPGFCGALGGAEEPPFVLLDTDAAGDRFFATYVLDPTRGSLHSAGTPVHFPRGGGAPGPDPSCWFEPDSICNGGVEPGLVFTGFLLVVGMGLMGAFLAHYVRHRLLHIQMVSGPNKIILTLDDITFLHPQGGSARKVVQGSRSSLAARSTSDVRSVPSQPSDGGNIGLYEGDWVWLKKFPGSQHIAIRPATKTAFSKLRELRHENVALYLGLFLGGGEGGSAAAGGGMLAVVSEHCTRGSLHDLLAQRDIKLDWMFKSSLLLDLIKGMRYLHHRGVAHGRLKSRNCVVDGRFVLKVTDHGHGRLLEAQKVLAEPPSAEDQLWTAPELLRDPALERRGTLAGDVFSLGIIMQEVVCRSSPYAMLELSAREVVQRVRSPPPLCRPSVSVDQAPAECIQLMKQCWAEQPELRPSLDRTFDQFKSINKGRKTNIIDSMLRMLEQYSSNLEGLIRERTEELELEKRKTDRLRAASLPSSVAEALKMGTPVEPEYFEEVTLYFSDIVGFTTISAMSEPIEVVDLLNDLYTLFDAIIGSHDVYKVETIGDAYMVASGLPQRNGQRHAAEIANMALDILSAVGSFRMRHMPEVPVRIRIGLHSGPCVAGVVGLTMPRYCLFGDTVNTASRMESTGLPYRIHVNMSTVRILRALDEGFQTEVRGRTELKGKGAEDTYWLVGXXXXXXXXPIPKPPDLQPGASNHGISLQEIPLDRRQKLEKARPGQFSGK

SEQ ID NO: 10 - protein, 1093 aa, Monodelphis domestica
MLVPSINGLFHHPPWCFPPLPLPLFFLFLLLLLPVPVLPATFTIGVLGPWSCDPIFSRARPDLAARLAATRMNHDQALEGGPWFEVILLPEPCRTSGSLGALSPSLARVSGLVGPVNPAACHPAELLAQEAGVPLVPWGCPQGKARTTAPALPLALDALYALLRAFHWAKVALITAPQDLWVEAGQALAGGLRSRGLPVAMVTSLETTDLESAKNALKRVRDGPKVKVLIMVMHSVLLGGEEQRLLLEAAEELGLVEGTMVFLPFDTLHYALPPGPEALRPITNSSRLRKAHDAVLTLTRYCPKGSVSASLRQAQEHRELPLDLKPQQVSPLFGTIYDAIYLLAGAVAGAQVAGGGGWVSGAAVARHIPNTLVSGFCGDLGGTKEPPFVLLDTDGMRDQLLPTYTLDPAQGVLHHAGNPIHFPHGGQGPGPDPPCWFDPNVICSGGIEPRFILLVILIIIGGGLVVATLAYYVRRQLLHAQMVSGPNKMILTLEDITFFPRQGSSSRKATEGSRSSLIAHSASDMRSIPSQPPDNSNIGMYEGDWVWLKKFPGEHYTEIRPATKMAFSKLRELRHENVAVQMGLFLAGSMEGAAAGGLGGGILAVVSEYCSRGSLQDLLIQRDIKLDWMFKSSLLLDLIKGLRYLHHRGVAHGRLKSRNCVVDGRFVLKITDHAHGRLLEAQRVSLEPPQAEDRLWTAPELLRNEALERQGTLQGDVFSVGIIMQEVVCRCEPYAMLELTPEEIIQKVQSPPPMCRPSVSVDQAPMECIQLMKQCWAEQPDLRPNMDTTFDLFKNINKGRKTNIIDSMLRMLEQYSSNLEDLIRERTEELELEKQKTDKLLTQMLPPSVAEALKLGIPVEPEYFEEVTLYFSDIVGFTTISAMSEPIEVVDLLNDLYTLFDAIIGSHDVYKVETIGDAYMVASGLPKRNGQRHAAEIANMSLDILSSVGSFRMRHMPEVPVRIRIGLHSGPCVAGVVGLTMPRYCLFGDTVNTASRMESTGLPYRIHVNLSTVKILQGLNEGFQIEIRGRTELKGKGVEDTYWLVGRKGFDKPIPIPPDLLPGASNHGISLQEIPEDRRKKLEKARPGQPLGK

SEQ ID NO: 11 - protein, 862 aa, Equus caballus
MVMHSVLLGGEEQRCLLEAAEELGLADGSLVFLPFDTLHYALSPGPEALAVLANNSQLRRAHDAVLTLTRHCPLGGSVLDSLRRAQEHQELPSDLNLQQVSPLFGTIYDAVYLLAGGVARARAAAGGSWVSGAAVAHHVRDAQVPGFCGALGGAEEPQFVLLDTDAAGDRLFATYMLDPTRGSLWSAGTPVHFPRGGRGPGPDPWCWFDPDDICNGGVEPRLVFIGFLLAVGMGLAGVFLAHYVRHRLLHIQMASGPNKIILTLDDITFLHPQGGSSRKVIQGSRSSLAARSVSDIRSVPSQPMDSSNIGLYEGDWVWLKKFPGDQHIAIRPATKTAFSKLRELRHENVALYLGLFLAGGSSGAAAPREGMLAVVSEHCARGSLHDLLAQRDIKLDWMFKSSLLLDLIKGMRYLHHRGVAHGRLKSRNCVVDGRFVLKVTDHGHGRLLEAQKVLPEPPSAEDQLWTAPELLRDPALERQGTLAGDVFSLGIIIQEVVCRSTPYAMLELTPEEVVQRLQSPPPLCRPSVSMDQAPMECIQLMKQCWAEQPDLRPSMDRTFDLFKSINKGRKTNIIDSMLRMLEQYSSNLEDLIRERTEELELEKQKTDRLLTQMLPPSVAEALKMGTPVEPEYFEEVTLYFSDIVGFTTISAMSEPIEVVDLLNDLYTLFDAIIGSHDVYKVETIGDAYMVASGLPQRNGQRHAAEIANMALDILSAVGSFRMRHMPEVPVRIRIGLHSGPCVAGVVGLTMPRYCLFGDTVNTASRMESTGLPYRIHVNMSTVRILRALDEGFQVEVRGRTELKGKGVEDTYWLVGRRGFNKPIPKPPDLQPGASNHGISLQEIPPERRQKLEKARPGQFSGK

SEQ ID NO: 12 - DNA, 292 bp, Homo sapiens
gggccccagaagcctggtggttgtttgtccttctcaggggaaaagtgaggcggccccttggaggaaggggccgggcagaatgatctaatcggattccaagcagctcaggggattgtctttttctagcaccttcttgccactcctaagcgtcctccgtgaccccggctgggatttagcctggtgctgtgtcagccccggtctcccaggggcttcccagtggtccccaggaaccctcgacagggcccggtctctctcgtccagcaagggcagggacgggccacaggccaagggc

SEQ ID NO: 13 - DNA, 953 bp, Artificial Sequence
  hybrid CBA/CMV promoter
aattcggtaccctagttattaatagtaatcaattacggggtcattagttcatagcccatatatggagttccgcgttacataacttacggtaaatggcccgcctggctgaccgcccaacgacccccgcccattgacgtcaataatgacgtatgttcccatagtaacgccaatagggactttccattgacgtcaatgggtggactatttacggtaaactgcccacttggcagtacatcaagtgtatcatatgccaagtacgccccctattgacgtcaatgacggtaaatggcccgcctggcattatgcccagtacatgaccttatgggactttcctacttggcagtacatctacgtattagtcatcgctattaccatggtcgaggtgagccccacgttctgcttcactctccccatctcccccccctccccacccccaattttgtatttatttattttttaattattttgtgcagcgatgggggcggggggggggggggggcgcgcgccaggcggggcggggcggggcgaggggcggggcggggcgaggcggagaggtgcggcggcagccaatcagagcggcgcgctccgaaagtttccttttatggcgaggcggcggcggcggcggccctataaaaagcgaagcgcgcggcgggcgggagtcgctgcgacgctgccttcgccccgtgccccgctccgccgccgcctcgcgccgcccgccccggctctgactgaccgcgttactcccacaggtgagcgggcgggacggcccttctcctccgggctgtaattagcgcttggtttaatgacggcttgtttcttttctgtggctgcgtgaaagccttgaggggctccgggagctagagcctctgctaaccatgttcatgccttcttctttttcctacagctcctgggcaacgtgctggttattgtgctgtctcatcattttggcaaag

SEQ ID NO: 14 - DNA, 36 bp, Artificial Sequence
  Forward Primer
aaaagcggccgcatgagcgcttggctcctgccagcc

SEQ ID NO: 15 - DNA, 36 bp, Artificial Sequence
  Reverse Primer
aaaagcggccgctcacttcccagtaaactggcctgg

SEQ ID NO: 16 - DNA, 24 bp, Artificial Sequence
  Forward Primer
gacccttcctgctggttcgatcca

SEQ ID NO: 17 - DNA, 25 bp, Artificial Sequence
  Reverse Primer
ctgcatgtgtagcagcctgtgcctc

SEQ ID NO: 18 - protein, 992 aa, Artificial Sequence
  Consensus Sequence
MSAAGGLGCPRAPSIPRLLLLLLLSLSAVFVGVLGPWACDPIFARARPDIAARLAARLNALDGGPRFEVALLPEPCTPGSLGAVSSASRVSGLVGPVNPAACRPAELLAQEAGVALVPWGVPGTRAAGTTAPVTPAADALYLLRAFRWAVALITAPQDLWVEAGALSTALRARGLPVALVTSMEVRVIMVMGSVLLGGEEQRLLEAAEELALDGSLVFLPFDTLHWALSPGPDAIANSSQLRKAHDAVLTLTRCPGGSVDSLRRAQEHELPLDLNLQVSPLFGTIYDAVFLLAGGTATAGGGWVSGAAVARIRDAVGFCGLGEEPSFVLIDTDASGDQLFATHLLDPGSAGTPMHFPKGGAPGPDPSCWFDPDICNGGVEPLVFIGFLLVIGMGLGAFLAFLAHYRHRLLHIQMSGPNKIILTLDDITFLHPGGSRKVQGSRSSLARSSDIRSISQDTNIGLYEGDWVWLKKFPGDHIAIRPATKAFSKIRELRHENVALYLGLFLAGAGAPAPGEGILAVVSEHCARGSLDLLAQRDIKLDWMFKSSLLLDLIKGIRYLHHRGVAHGRLKSRNCVVDGRFVLKVTDHGHGRLLEAQRVLPEPPSAEDQLWTAPELLRDPLERRRGTLAGDVFSLAIIMQEVVCRSPYAMLELTPEEVIRVSPPPLCRPVSIDQAPMECIQLMQVWAEPELRPSMDTFDLFKSINKGRKNIIDSMLRMLEQYSSNLEDLIRERTEELEEEKQKTDRLLTQMLPPSVAEALKMGTVEPEYFEEVTLYFSDIVGFTTISAMSEPIEVVDLLNDLYTLFDAIIGAHDVYKVETIGDAYMVASGLPQRNGRHAAEIANMALDILSAVGSFRFRMRHMPEVPVRIRIGLHSGPCVAGVVGLTMPRYCLFGDTVNTASMESTGLPYRIHVNSTVILALGFERGRTELKGKGEDTYWLVGRGFNKPIPKPPDLQPGASNHGISLHGISLEIPPDRRKLEKARPGQFSGK